European Patent Application EP 4 303 300 A1, published January 10, 2024. Title: GENE FOR EFFICIENTLY EXPRESSING HYALURONIC ACID HYDROLASE AND EXPRESSION METHOD THEREOF. Applicant: BLOOMAGE BIOTECHNOLOGY CORPORATION LIMITED. The sequence listing filed with the application follows.

SEQUENCE LISTING (7 sequences)

SEQ ID NO: 1 - DNA, 1074 bp, Artificial sequence
  Description of Artificial Sequence: artificially synthesized sequence
atgatcccacccgcacgtgactcgcttatgtttgtctttgcgactgcggtaatcgctagttttttcggtagcgcaaagacactacgcggctcttccccacagcaattcgacgtatactggaatgtgccaactttcatgtgtcacaagcacggtatgaaatttgaagagctgaaagatttcggtatacaccagaacgcaatggatatgtttcgcggcgaagaaattgcgattctttatgaccctggcatgtttcccgcccttctagtagataaagatggatacgtcactaaacggaacggtggggtgccgcaagaggggaacctcaaggaacatttagaaacctttagaaagcatctgacgacacaaattccggacgagagctttagcgggataggaatcatagactttgagagttggagaccgattttcaggcagaactgggcgtcactcgagccctataaaactttgtccataaagttggagagggaaaaacacccattttggtcggaggcagctgtgaagaaggaggccaaacgtcgattcgagaaatccgggcgaatatttatggaggaaaccctcaaaatggccaaaaaactaagaccgaaagcaaagtggggctattatgggtatccccactgtttcaatcaaacccctggacagcagtcggttcactgcaatcggcaaacgatgatggaaaatgacggtatgagttggctgtttacactcgaagacgttcatgctcccagcgtttacctacgattggaaatcaaggaggatgaccggccttcattcgtgaaaggccgggtttccgaggccttaaggttagccgctaaatcgtcttcaaaacaacgtatcctaccttactactggttcatttatcaggataagaaggatgagttcttaacggaaaaggatacacaaaacactataaatatgatcgctaatctgggatctaatggtttcataatttggggatctagtgacgatgtcaacacggaacgcaaatgcaaggatttacagcaatacgtaaaggaagtcttgggcccagcgattaagaagttcacccttcattga

SEQ ID NO: 2 - protein, 357 aa, Artificial sequence
  Description of Artificial Sequence: artificially synthesized sequence
MIPPARDSLMFVFATAVIASFFGSAKTLRGSSPQQFDVYWNVPTFMCHKHGMKFEELKDFGIHQNAMDMFRGEEIAILYDPGMFPALLVDKDGYVTKRNGGVPQEGNLKEHLETFRKHLTTQIPDESFSGIGIIDFESWRPIFRQNWASLEPYKTLSIKLEREKHPFWSEAAVKKEAKRRFEKSGRIFMEETLKMAKKLRPKAKWGYYGYPHCFNQTPGQQSVHCNRQTMMENDGMSWLFTLEDVHAPSVYLRLEIKEDDRPSFVKGRVSEALRLAAKSSSKQRILPYYWFIYQDKKDEFLTEKDTQNTINMIANLGSNGFIIWGSSDDVNTERKCKDLQQYVKEVLGPAIKKFTLH

SEQ ID NO: 3 - DNA, 72 bp, Artificial sequence
  Description of Artificial Sequence: artificially synthesized sequence
atcccacccgcacgtgactcgcttatgtttgtctttgcgactgcggtaatcgctagttttttcggtagcgca

SEQ ID NO: 4 - DNA, 1020 bp, Artificial sequence
  Description of Artificial Sequence: artificially synthesized sequence
atgaagacactacgcggctcttccccacagcaattcgacgtatactggaatgtgccaactttcatgtgtcacaagcacggtatgaaatttgaagagctgaaagatttcggtatacaccagaacgcaatggatatgtttcgcggcgaagaaattgcgattctttatgaccctggcatgtttcccgcccttctagtagataaagatggatacgtcactaaacggaacggtggggtgccgcaagaggggaacctcaaggaacatttagaaacctttagaaagcatctgacgacacaaattccggacgagagctttagcgggataggaatcatagactttgagagttggagaccgattttcaggcagaactgggcgtcactcgagccctataaaactttgtccataaagttggagagggaaaaacacccattttggtcggaggcagctgtgaagaaggaggccaaacgtcgattcgagaaatccgggcgaatatttatggaggaaaccctcaaaatggccaaaaaactaagaccgaaagcaaagtggggctattatgggtatccccactgtttcaatcaaacccctggacagcagtcggttcactgcaatcggcaaacgatgatggaaaatgacggtatgagttggctgtttacactcgaagacgttcatgctcccagcgtttacctacgattggaaatcaaggaggatgaccggccttcattcgtgaaaggccgggtttccgaggccttaaggttagccgctaaatcgtcttcaaaacaacgtatcctaccttactactggttcatttatcaggataagaaggatgagttcttaacggaaaaggatacacaaaacactataaatatgatcgctaatctgggatctaatggtttcataatttggggatctagtgacgatgtcaacacggaacgcaaatgcaaggatttacagcaatacgtaaaggaagtcttgggcccagcgattaagaagttcacccttcatcaccaccatcatcatcattga

SEQ ID NO: 5 - protein, 339 aa, Artificial sequence
  Description of Artificial Sequence: artificially synthesized sequence
MKTLRGSSPQQFDVYWNVPTFMCHKHGMKFEELKDFGIHQNAMDMFRGEEIAILYDPGMFPALLVDKDGYVTKRNGGVPQEGNLKEHLETFRKHLTTQIPDESFSGIGIIDFESWRPIFRQNWASLEPYKTLSIKLEREKHPFWSEAAVKKEAKRRFEKSGRIFMEETLKMAKKLRPKAKWGYYGYPHCFNQTPGQQSVHCNRQTMMENDGMSWLFTLEDVHAPSVYLRLEIKEDDRPSFVKGRVSEALRLAAKSSSKQRILPYYWFIYQDKKDEFLTEKDTQNTINMIANLGSNGFIIWGSSDDVNTERKCKDLQQYVKEVLGPAIKKFTLHHHHHHH

SEQ ID NO: 6 - DNA, 29 bp, Artificial sequence
  Description of Artificial Sequence: artificially synthesized sequence
ccggaattcatgaagacactacgcggctc

SEQ ID NO: 7 - DNA, 51 bp, Artificial sequence
  Description of Artificial Sequence: artificially synthesized sequence
atttgcggccgctcaatgatgatgatggtggtgatgaagggtgaacttctt